European Patent Application EP 4 046 635 A9, published October 11, 2023. Title: COMPOSITION FOR PREVENTING HAIR LOSS OR PROMOTING HAIR GROWTH COMPRISING RIP KINASE INHIBITOR. Applicant: STEMORE CO., LTD. The sequence listing filed with the application follows.

SEQUENCE LISTING (4 sequences)

SEQ ID NO: 1 - RNA, 19 nt, Artificial Sequence
  RIPK1 siRNA siRNA No (19766-1)
guccuuguguuaccacaga

SEQ ID NO: 2 - RNA, 19 nt, Artificial Sequence
  RIPK1 siRNA siRNA No (19766-1)
ucugugguaacacaaggac

SEQ ID NO: 3 - RNA, 19 nt, Artificial Sequence
  RIPK3 siRNA siRNA No (56532-1)
cgagugaugucuacagcuu

SEQ ID NO: 4 - RNA, 19 nt, Artificial Sequence
  RIPK3 siRNA siRNA No (56532-1)
aagcuguagacaucacucg